European Patent Specification EP 3 775 171 B1, published January 3, 2024. Title: METHODS OF TREATING MINIMAL RESIDUAL CANCER. Applicant: ICAHN SCHOOL OF MEDICINE AT MOUNT SINAI. The sequence listing filed with the application follows.

SEQUENCE LISTING (16 sequences)

SEQ ID NO: 1 - protein, 431 aa, Homo sapiens
MHVRSLRAAAPHSFVALWAPLFLLRSALADFSLDNEVHSSFIHRRLRSQERREMQREILSILGLPHRPRPHLQGKHNSAPMFMLDLYNAMAVEEGGGPGGQGFSYPYKAVFSTQGPPLASLQDSHFLTDADMVMSFVNLVEHDKEFFHPRYHHREFRFDLSKIPEGEAVTAAEFRIYKDYIRERFDNETFRISVYQVLQEHLGRESDLFLLDSRTLWASEEGWLVFDITATSNHWVVNPRHNLGLQLSVETLDGQSINPKLAGLIGRHGPQNKQPFMVAFFKATEVHFRSIRSTGSKQRSQNRSKTPKNQEALRMANVAENSSSDQRQACKKHELYVSFRDLGWQDWIIAPEGYAAYYCEGECAFPLNSYMNATNHAIVQTLVHFINPETVPKPCCAPTQLNAISVLYFDDSSNVILKKYRNMVVRACGCH

SEQ ID NO: 2 - protein, 139 aa, Homo sapiens
STGSKQRSQNRSKTPKNQEALRMANVAENSSSDQRQACKKHELYVSFRDLGWQDWIIAPEGYAAYYCEGECAFPLNSYMNATNHAIVQTLVHFINPETVPKPCCAPTQLNAISVLYFDDSSNVILKKYRNMVVRACGCH

SEQ ID NO: 3 - protein, 139 aa, Homo sapiens
  misc_feature (33)..(33): Xaa can be any naturally occurring amino acid
  misc_feature (37)..(37): Xaa can be any naturally occurring amino acid
  misc_feature (60)..(60): Xaa can be any naturally occurring amino acid
  misc_feature (65)..(65): Xaa can be any naturally occurring amino acid
  misc_feature (86)..(87): Xaa can be any naturally occurring amino acid
  misc_feature (89)..(89): Xaa can be any naturally occurring amino acid
  misc_feature (91)..(91): Xaa can be any naturally occurring amino acid
  misc_feature (93)..(94): Xaa can be any naturally occurring amino acid
  misc_feature (110)..(110): Xaa can be any naturally occurring amino acid
  misc_feature (114)..(114): Xaa can be any naturally occurring amino acid
  misc_feature (120)..(120): Xaa can be any naturally occurring amino acid
  misc_feature (128)..(128): Xaa can be any naturally occurring amino acid
  misc_feature (132)..(132): Xaa can be any naturally occurring amino acid
  misc_feature (134)..(134): Xaa can be any naturally occurring amino acid
STGSKQRSQNRSKTPKNQEALRMANVAENSSSXQRQXCKKHELYVSFRDLGWQDWIIAPXGYAAXYCEGECAFPLNSYMNATNHAXXQXLXHXXNPETVPKPCCAPTQLXAISXLYFDDXSNVILKKXRNMXVXACGCH

SEQ ID NO: 4 - protein, 139 aa, Homo sapiens
STGSKQRSQNRSKTPKNQEALRMANVAENSSSDQRQACKKHELYVSFRDLGWQDWIIAPEGYAAYYCEGECAFPLNSYMNATNHAIVQTLVHVINPETVPKPCCAPTQLGAISVLYFDDSSNVILKKYRNMVVRACGCH

SEQ ID NO: 5 - protein, 139 aa, Homo sapiens
STGSKQRSQNRSKTPKNQEALRMANVAENSSSDQRQACKKHELYVSFRDLGWQDWIIAPEGYAAGYCEGECAFPLNSYMNATNHALVQALVHFINPETVPKPCCAPTQLGAISVLYFDDSSNVILKKYRNMVVRACGCH

SEQ ID NO: 6 - protein, 139 aa, Homo sapiens
STGSKQRSQNRSKTPKNQEALRMANVAENSSSDQRQACKKHELYVSFRDLGWQDWIIAPEGYAAGYCEGECAFPLNSYMNATNHALVQTLVHFINPETVPKPCCAPTQLGAISVLYFDDSSNVILKKFRNMVVRACGCH

SEQ ID NO: 7 - protein, 139 aa, Homo sapiens
STGSKQRSQNRSKTPKNQEALRMANVAENSSSDQRQACKKHELYVSFRDLGWQDWIIAPEGYAAGYCEGECAFPLNSYMNATNHALVQTLVHFINPETVPKPCCAPTQLGAISVLYFDDSSNVILKKWRNMVVRACGCH

SEQ ID NO: 8 - protein, 139 aa, Homo sapiens
STGSKQRSQNRSKTPKNQEALRMANVAENSSSDQRQACKKHELYVSFRDLGWQDWIIAPEGYAAGYCEGECAFPLNSYMNATNHALVQTLVHVINPETVPKPCCAPTQLGAISVLYFDDSSNVILKKWRNMVVRACGCH

SEQ ID NO: 9 - protein, 139 aa, Homo sapiens
STGSKQRSQNRSKTPKNQEALRMANVAENSSSDQRQACKKHELYVSFRDLGWQDWIIAPEGYAAGYCEGECAFPLNSYMNATNHAIVQALVHFINPETVPKPCCAPTQLGAISVLYFDDSSNVILKKFRNMVVRACGCH

SEQ ID NO: 10 - protein, 139 aa, Homo sapiens
STGSKQRSQNRSKTPKNQEALRMANVAENSSSDQRQACKKHELYVSFRDLGWQDWIIAPEGYAAGYCEGECAFPLNSYMNATNHALVQTLVHFINPETVPKPCCAPTQLGAISVLYFDDSSNVILKKYRNMVVRACGCH

SEQ ID NO: 11 - protein, 139 aa, Homo sapiens
STGSKQRSQNRSKTPKNQEALRMANVAENSSSDQRQACKKHELYVSFRDLGWQDWIIAPEGYAAGYCEGECAFPLNSYMNATNHAIVQTLVHFINPETVPKPCCAPTQLNAISMLYFDDSSNVILKKYRNMVVRACGCH

SEQ ID NO: 12 - protein, 402 aa, Homo sapiens
DFSLDNEVHSSFIHRRLRSQERREMQREILSILGLPHRPRPHLQGKHNSAPMFMLDLYNAMAVEEGGGPGGQGFSYPYKAVFSTQGPPLASLQDSHFLTDADMVMSFVNLVEHDKEFFHPRYHHREFRFDLSKIPEGEAVTAAEFRIYKDYIRERFDNETFRISVYQVLQEHLGRESDLFLLDSRTLWASEEGWLVFDITATSNHWVVNPRHNLGLQLSVETLDGQSINPKLAGLIGRHGPQNKQPFMVAFFKATEVHFRSIRSTGSKQRSQNRSKTPKNQEALRMANVAENSSSDQRQACKKHELYVSFRDLGWQDWIIAPEGYAAYYCEGECAFPLNSYMNATNHAIVQTLVHVINPETVPKPCCAPTQLGAISVLYFDDSSNVILKKYRNMVVRACGCH

SEQ ID NO: 13 - protein, 402 aa, Homo sapiens
DFSLDNEVHSSFIHRRLRSQERREMQREILSILGLPHRPRPHLQGKHNSAPMFMLDLYNAMAVEEGGGPGGQGFSYPYKAVFSTQGPPLASLQDSHFLTDADMVMSFVNLVEHDKEFFHPRYHHREFRFDLSKIPEGEAVTAAEFRIYKDYIRERFDNETFRISVYQVLQEHLGRESDLFLLDSRTLWASEEGWLVFDITATSNHWVVNPRHNLGLQLSVETLDGQSINPKLAGLIGRHGPQNKQPFMVAFFKATEVHFRSIRSTGSKQRSQNRSKTPKNQEALRMANVAENSSSDQRQACKKHELYVSFRDLGWQDWIIAPEGYAAGYCEGECAFPLNSYMNATNHALVQALVHFINPETVPKPCCAPTQLGAISVLYFDDSSNVILKKYRNMVVRACGCH

SEQ ID NO: 14 - protein, 402 aa, Homo sapiens
DFSLDNEVHSSFIHRRLRSQERREMQREILSILGLPHRPRPHLQGKHNSAPMFMLDLYNAMAVEEGGGPGGQGFSYPYKAVFSTQGPPLASLQDSHFLTDADMVMSFVNLVEHDKEFFHPRYHHREFRFDLSKIPEGEAVTAAEFRIYKDYIRERFDNETFRISVYQVLQEHLGRESDLFLLDSRTLWASEEGWLVFDITATSNHWVVNPRHNLGLQLSVETLDGQSINPKLAGLIGRHGPQNKQPFMVAFFKATEVHFRSIRSTGSKQRSQNRSKTPKNQEALRMANVAENSSSDQRQACKKHELYVSFRDLGWQDWIIAPEGYAAGYCEGECAFPLNSYMNATNHALVQTLVHFINPETVPKPCCAPTQLGAISVLYFDDSSNVILKKFRNMVVRACGCH

SEQ ID NO: 15 - protein, 402 aa, Homo sapiens
DFSLDNEVHSSFIHRRLRSQERREMQREILSILGLPHRPRPHLQGKHNSAPMFMLDLYNAMAVEEGGGPGGQGFSYPYKAVFSTQGPPLASLQDSHFLTDADMVMSFVNLVEHDKEFFHPRYHHREFRFDLSKIPEGEAVTAAEFRIYKDYIRERFDNETFRISVYQVLQEHLGRESDLFLLDSRTLWASEEGWLVFDITATSNHWVVNPRHNLGLQLSVETLDGQSINPKLAGLIGRHGPQNKQPFMVAFFKATEVHFRSIRSTGSKQRSQNRSKTPKNQEALRMANVAENSSSDQRQACKKHELYVSFRDLGWQDWIIAPEGYAAGYCEGECAFPLNSYMNATNHALVQTLVHFINPETVPKPCCAPTQLGAISVLYFDDSSNVILKKWRNMVVRACGCH

SEQ ID NO: 16 - protein, 402 aa, Homo sapiens
DFSLDNEVHSSFIHRRLRSQERREMQREILSILGLPHRPRPHLQGKHNSAPMFMLDLYNAMAVEEGGGPGGQGFSYPYKAVFSTQGPPLASLQDSHFLTDADMVMSFVNLVEHDKEFFHPRYHHREFRFDLSKIPEGEAVTAAEFRIYKDYIRERFDNETFRISVYQVLQEHLGRESDLFLLDSRTLWASEEGWLVFDITATSNHWVVNPRHNLGLQLSVETLDGQSINPKLAGLIGRHGPQNKQPFMVAFFKATEVHFRSIRSTGSKQRSQNRSKTPKNQEALRMANVAENSSSDQRQACKKHELYVSFRDLGWQDWIIAPEGYAAGYCEGECAFPLNSYMNATNHALVQTLVHVINPETVPKPCCAPTQLGAISVLYFDDSSNVILKKWRNMVVRACGCH